European Patent Specification EP 4 114 973 B1, published August 13, 2025. Title: Hydrolysis-based probe and method for STR genotyping. Applicant: Universiteit Gent. The sequence listing filed with the application follows.

SEQUENCE LISTING (14 sequences)

SEQ ID NO: 1 - DNA, 52 bp, Artificial sequence
  probe
ctgttcctcccttatttccctcattcattcattcattcattcattcaccatg

SEQ ID NO: 2 - DNA, 56 bp, Artificial sequence
  probe
ctgttcctcccttatttccctcattcattcattcattcattcattcattcaccatg

SEQ ID NO: 3 - DNA, 60 bp, Artificial sequence
  probe
ctgttcctcccttatttccctcattcattcattcattcattcattcattcattcaccatg

SEQ ID NO: 4 - DNA, 75 bp, Artificial sequence
  complementary to probe
acagactccatggtgaatgaatgaatgaatgaatgaatgagggaaataagggaggaacaggccaatgggaatcac

SEQ ID NO: 5 - DNA, 79 bp, Artificial sequence
  complementary to probe
acagactccatggtgaatgaatgaatgaatgaatgaatgaatgagggaaataagggaggaacaggccaatgggaatcac

SEQ ID NO: 6 - DNA, 83 bp, Artificial sequence
  complementary to probe
acagactccatggtgaatgaatgaatgaatgaatgaatgaatgaatgagggaaataagggaggaacaggccaatgggaatcac

SEQ ID NO: 7 - DNA, 21 bp, Artificial sequence
  primer
gtgattcccattggcctgttc

SEQ ID NO: 8 - DNA, 22 bp, Artificial sequence
  primer
attcctgtgggctgaaaagctc

SEQ ID NO: 9 - DNA, 52 bp, Artificial sequence; identical to SEQ ID NO: 1
  probe

SEQ ID NO: 10 - DNA, 56 bp, Artificial sequence; identical to SEQ ID NO: 2
  probe

SEQ ID NO: 11 - DNA, 60 bp, Artificial sequence; identical to SEQ ID NO: 3
  probe

SEQ ID NO: 12 - DNA, 60 bp, Artificial sequence; identical to SEQ ID NO: 3
  probe

SEQ ID NO: 13 - DNA, 67 bp, Artificial sequence
  probe
ctgttcctcccttatttccctcattcattcatcattcattcattcattcattcattcattcaccatg

SEQ ID NO: 14 - DNA, 64 bp, Artificial sequence
  probe
ctgttcctcccttatttccctcattcattcattcattcattcattcattcattcattcaccatg